European Patent Application EP 4 378 483 A1, published June 5, 2024. Title: USE OF ST-TYPE LIPID COMPOUNDS IN PREPARATION OF NUCLEIC ACID DELIVERY REAGENT AND RELATED PRODUCT. Applicant: INSTITUTE OF BASIC MEDICAL SCIENCES CHINESE ACADEMY OF MEDICAL SCIENCES. The sequence listing filed with the application follows.

SEQUENCE LISTING (7 sequences)

SEQ ID NO: 1 - RNA, 25 nt, synthetic construct
  source 1..25: mol_type = other RNA
tccggaatgattgggcgtaaagcgt

SEQ ID NO: 2 - RNA, 50 nt, synthetic construct
  source 1..50: mol_type = other RNA
gtcgtatccagtgcacgctccgaggtattcgcactggatacgacacgctt

SEQ ID NO: 3 - RNA, 21 nt, synthetic construct
  source 1..21: mol_type = other RNA
tcgcgctccggaatgattggg

SEQ ID NO: 4 - RNA, 16 nt, synthetic construct
  source 1..16: mol_type = other RNA
gtgcacgctccgaggt

SEQ ID NO: 5 - RNA, 53 nt, synthetic construct
  source 1..53: mol_type = other RNA
gtcgtatccagtgcagggtccgaggtattcgcactggatacgacaaaaatatg

SEQ ID NO: 6 - RNA, 18 nt, synthetic construct
  source 1..18: mol_type = other RNA
gcgcgtcgtgaagcgttc

SEQ ID NO: 7 - RNA, 16 nt, synthetic construct
  source 1..16: mol_type = other RNA
gtgcagggtccgaggt